European Patent Specification EP 3 318 627 B1, published October 25, 2023. Title: CULTURE MEDIA FOR STEM CELLS. Applicant: KONINKLIJKE NEDERLANDSE AKADEMIE VAN WETENSCHAPPEN. Application PCT/IB2012/052950. The sequence listing filed with the application follows.

SEQUENCE LISTING (30 sequences)

SEQ ID NO: 1 - protein, 17 aa, Artificial Sequence
  DSL peptide
CDDYYYGFGCNKFCRPR

SEQ ID NO: 2 - DNA, 22 bp, Artificial Sequence
  Primer
gcagcattacctgctctacgtt

SEQ ID NO: 3 - DNA, 25 bp, Artificial Sequence
  Reverse primer
gcttgataagctgatgctgtaattt

SEQ ID NO: 4 - DNA, 8 bp, Artificial Sequence
  Probe
gcagccag

SEQ ID NO: 5 - DNA, 18 bp, Artificial Sequence
  forward primer
catggaccgcttcccata

SEQ ID NO: 6 - DNA, 19 bp, Artificial Sequence
  reverse primer
ggcacctgtctgtccacat

SEQ ID NO: 7 - DNA, 8 bp, Artificial Sequence
  Probe
tggctctg

SEQ ID NO: 8 - DNA, 18 bp, Artificial Sequence
  Forward primer
cagccaacgctgcttctc

SEQ ID NO: 9 - DNA, 18 bp, Artificial Sequence
  Reverse primer
tggcatggaattgacagc

SEQ ID NO: 10 - DNA, 8 bp, Artificial Sequence
  Probe
cctcctgg

SEQ ID NO: 11 - DNA, 21 bp, Artificial Sequence
  Forward primer
ccgctactggtgtaatgatgg

SEQ ID NO: 12 - DNA, 22 bp, Artificial Sequence
  Reverse primer
catcagcgatgttatcttgcag

SEQ ID NO: 13 - DNA, 8 bp, Artificial Sequence
  Probe
aggagcag

SEQ ID NO: 14 - DNA, 19 bp, Artificial Sequence
  Forward primer
gccagctcatcaaggacag

SEQ ID NO: 15 - DNA, 21 bp, Artificial Sequence
  Reverse primer
gcaggcatcgtagtagtgctg

SEQ ID NO: 16 - DNA, 8 bp, Artificial Sequence
  Probe
ttgcccag

SEQ ID NO: 17 - DNA, 24 bp, Artificial Sequence
  Forward primer
tgaccttgatttattttgcatacc

SEQ ID NO: 18 - DNA, 20 bp, Artificial Sequence
  Reverse primer
cgagcaagacgttcagtcct

SEQ ID NO: 19 - DNA, 22 bp, Artificial Sequence
  Forward primer
gcttgccacaacttcctaagat

SEQ ID NO: 20 - DNA, 22 bp, Artificial Sequence
  Reverse primer
tcagtttagtcatggtggacga

SEQ ID NO: 21 - DNA, 8 bp, Artificial Sequence
  Probe
ggtggtgg

SEQ ID NO: 22 - DNA, 18 bp, Artificial Sequence
  Forward primer
tgtggaaccgggaagatg

SEQ ID NO: 23 - DNA, 21 bp, Artificial Sequence
  Reverse primer
gaccacaggtatggttctgga

SEQ ID NO: 24 - DNA, 8 bp, Artificial Sequence
  Probe
tggtggag

SEQ ID NO: 25 - DNA, 21 bp, Artificial Sequence
  Forward primer
cgatccagaaagatgatggtc

SEQ ID NO: 26 - DNA, 19 bp, Artificial Sequence
  Reverse primer
cggaagcctctgtctttcc

SEQ ID NO: 27 - DNA, 8 bp, Artificial Sequence
  Probe
ggatggag

SEQ ID NO: 28 - DNA, 19 bp, Artificial Sequence
  Forward primer
tcctcctcagaccgctttt

SEQ ID NO: 29 - DNA, 21 bp, Artificial Sequence
  Reverse primer
cctggttcatcatcgctaatc

SEQ ID NO: 30 - DNA, 8 bp, Artificial Sequence
  Probe
actcccag